European Patent Application EP 4 729 615 A1, published April 22, 2026. Title: 靶向MMP7的siRNA、siRNA缀合物及其医药用途. Applicant: 上海拓界生物医药科技有限公司. Application WO. The sequence listing filed with the application follows.

SEQUENCE LISTING (427 sequences)

SEQ ID NO: 1 - RNA, 19 nt, Homo sapiens
  source 1..19: mol_type = mRNA
tgggtagatgtcaataaat

SEQ ID NO: 2 - RNA, 19 nt, Homo sapiens
  source 1..19: mol_type = mRNA
tgactcagaaacaaaaaat

SEQ ID NO: 3 - RNA, 19 nt, Homo sapiens
  source 1..19: mol_type = mRNA
attcaagaaagaaatagaa

SEQ ID NO: 4 - RNA, 19 nt, Homo sapiens
  source 1..19: mol_type = mRNA
gactcagaaacaaaaaata

SEQ ID NO: 5 - RNA, 19 nt, Homo sapiens
  source 1..19: mol_type = mRNA
caacagtttagaagccaaa

SEQ ID NO: 6 - RNA, 19 nt, Homo sapiens
  source 1..19: mol_type = mRNA
caattatgtcacccttttt

SEQ ID NO: 7 - RNA, 19 nt, Homo sapiens
  source 1..19: mol_type = mRNA
gtgggtagatgtcaataaa

SEQ ID NO: 8 - RNA, 19 nt, Homo sapiens
  source 1..19: mol_type = mRNA
gggtagatgtcaataaata

SEQ ID NO: 9 - RNA, 19 nt, Homo sapiens
  source 1..19: mol_type = mRNA
ggtagatgtcaataaatgt

SEQ ID NO: 10 - RNA, 19 nt, Homo sapiens
  source 1..19: mol_type = mRNA
caaataaataaaatgttta

SEQ ID NO: 11 - RNA, 19 nt, synthetic construct
  source 1..19: mol_type = other RNA; note = The nucleotide modifications are shown in Table 1B
tgggtagatgtcaataaat

SEQ ID NO: 12 - RNA, 19 nt, synthetic construct
  source 1..19: mol_type = other RNA; note = The nucleotide modifications are shown in Table 1B
tgactcagaaacaaaaaat

SEQ ID NO: 13 - RNA, 19 nt, synthetic construct
  source 1..19: mol_type = other RNA; note = The nucleotide modifications are shown in Table 1B
attcaagaaagaaatagaa

SEQ ID NO: 14 - RNA, 19 nt, synthetic construct
  source 1..19: mol_type = other RNA; note = The nucleotide modifications are shown in Table 1B
gactcagaaacaaaaaata

SEQ ID NO: 15 - RNA, 19 nt, synthetic construct
  source 1..19: mol_type = other RNA; note = The nucleotide modifications are shown in Table 1B
gactcagaaacaaaaaata

SEQ ID NO: 16 - RNA, 19 nt, synthetic construct
  source 1..19: mol_type = other RNA; note = The nucleotide modifications are shown in Table 1B
caacagtttagaagccaaa

SEQ ID NO: 17 - RNA, 19 nt, synthetic construct
  source 1..19: mol_type = other RNA; note = The nucleotide modifications are shown in Table 1B
caacagtttagaagccaaa

SEQ ID NO: 18 - RNA, 19 nt, synthetic construct
  source 1..19: mol_type = other RNA; note = The nucleotide modifications are shown in Table 1B
caattatgtcacccttttt

SEQ ID NO: 19 - RNA, 19 nt, synthetic construct
  source 1..19: mol_type = other RNA; note = The nucleotide modifications are shown in Table 1B
caattatgtcacccttttt

SEQ ID NO: 20 - RNA, 19 nt, synthetic construct
  source 1..19: mol_type = other RNA; note = The nucleotide modifications are shown in Table 1B
gtgggtagatgtcaataaa

SEQ ID NO: 21 - RNA, 19 nt, synthetic construct
  source 1..19: mol_type = other RNA; note = The nucleotide modifications are shown in Table 1B
gtgggtagatgtcaataaa

SEQ ID NO: 22 - RNA, 19 nt, synthetic construct
  source 1..19: mol_type = other RNA; note = The nucleotide modifications are shown in Table 1B
gggtagatgtcaataaata

SEQ ID NO: 23 - RNA, 19 nt, synthetic construct
  source 1..19: mol_type = other RNA; note = The nucleotide modifications are shown in Table 1B
gggtagatgtcaataaata

SEQ ID NO: 24 - RNA, 19 nt, synthetic construct
  source 1..19: mol_type = other RNA; note = The nucleotide modifications are shown in Table 1B
ggtagatgtcaataaatgt

SEQ ID NO: 25 - RNA, 19 nt, synthetic construct
  source 1..19: mol_type = other RNA; note = The nucleotide modifications are shown in Table 1B
ggtagatgtcaataaatgt

SEQ ID NO: 26 - RNA, 19 nt, synthetic construct
  source 1..19: mol_type = other RNA; note = The nucleotide modifications are shown in Table 1B
caaataaataaaatgttta

SEQ ID NO: 27 - RNA, 19 nt, synthetic construct
  source 1..19: mol_type = other RNA; note = The nucleotide modifications are shown in Table 1B
caaataaataaaatgttta

SEQ ID NO: 28 - RNA, 19 nt, synthetic construct
  source 1..19: mol_type = other RNA; note = The nucleotide modifications are shown in Table 1b, with a ligand linked to the 5' end
tgggtagatgtcaataaat

SEQ ID NO: 29 - RNA, 19 nt, synthetic construct
  source 1..19: mol_type = other RNA; note = The nucleotide modifications are shown in Table 1b, with a ligand linked to the 5' end
tgactcagaaacaaaaaat

SEQ ID NO: 30 - RNA, 19 nt, synthetic construct
  source 1..19: mol_type = other RNA; note = The nucleotide modifications are shown in Table 1b, with a ligand linked to the 5' end
attcaagaaagaaatagaa

SEQ ID NO: 31 - RNA, 21 nt, Homo sapiens
  source 1..21: mol_type = mRNA
atttattgacatctacccact

SEQ ID NO: 32 - RNA, 21 nt, Homo sapiens
  source 1..21: mol_type = mRNA
attttttgtttctgagtcata

SEQ ID NO: 33 - RNA, 21 nt, Homo sapiens
  source 1..21: mol_type = mRNA
ttctatttctttcttgaatta

SEQ ID NO: 34 - RNA, 21 nt, Homo sapiens
  source 1..21: mol_type = mRNA
tattttttgtttctgagtcat

SEQ ID NO: 35 - RNA, 21 nt, Homo sapiens
  source 1..21: mol_type = mRNA
tttggcttctaaactgttggc

SEQ ID NO: 36 - RNA, 21 nt, Homo sapiens
  source 1..21: mol_type = mRNA
aaaaagggtgacataattgct

SEQ ID NO: 37 - RNA, 21 nt, Homo sapiens
  source 1..21: mol_type = mRNA
tttattgacatctacccactg

SEQ ID NO: 38 - RNA, 21 nt, Homo sapiens
  source 1..21: mol_type = mRNA
tatttattgacatctacccac

SEQ ID NO: 39 - RNA, 21 nt, Homo sapiens
  source 1..21: mol_type = mRNA
acatttattgacatctaccca

SEQ ID NO: 40 - RNA, 21 nt, Homo sapiens
  source 1..21: mol_type = mRNA
taaacattttatttatttgtg

SEQ ID NO: 41 - RNA, 21 nt, synthetic construct
  source 1..21: mol_type = other RNA; note = The nucleotide modifications are shown in Table 1B
atttattgacatctacccact

SEQ ID NO: 42 - RNA, 21 nt, synthetic construct
  source 1..21: mol_type = other RNA; note = The nucleotide modifications are shown in Table 1B
attttttgtttctgagtcata

SEQ ID NO: 43 - RNA, 21 nt, synthetic construct
  source 1..21: mol_type = other RNA; note = The nucleotide modifications are shown in Table 1B
ttctatttctttcttgaatta

SEQ ID NO: 44 - RNA, 21 nt, synthetic construct
  source 1..21: mol_type = other RNA; note = The nucleotide modifications are shown in Table 1B
tattttttgtttctgagtcat

SEQ ID NO: 45 - RNA, 21 nt, synthetic construct
  source 1..21: mol_type = other RNA; note = The nucleotide modifications are shown in Table 1B
tattttttgtttctgagtcat

SEQ ID NO: 46 - RNA, 21 nt, synthetic construct
  source 1..21: mol_type = other RNA; note = The nucleotide modifications are shown in Table 1B
tttggcttctaaactgttggc

SEQ ID NO: 47 - RNA, 21 nt, synthetic construct
  source 1..21: mol_type = other RNA; note = The nucleotide modifications are shown in Table 1B
tttggcttctaaactgttggc

SEQ ID NO: 48 - RNA, 21 nt, synthetic construct
  source 1..21: mol_type = other RNA; note = The nucleotide modifications are shown in Table 1B
aaaaagggtgacataattgct

SEQ ID NO: 49 - RNA, 21 nt, synthetic construct
  source 1..21: mol_type = other RNA; note = The nucleotide modifications are shown in Table 1B
aaaaagggtgacataattgct

SEQ ID NO: 50 - RNA, 21 nt, synthetic construct
  source 1..21: mol_type = other RNA; note = The nucleotide modifications are shown in Table 1B
tttattgacatctacccactg

SEQ ID NO: 51 - RNA, 21 nt, synthetic construct
  source 1..21: mol_type = other RNA; note = The nucleotide modifications are shown in Table 1B
tttattgacatctacccactg

SEQ ID NO: 52 - RNA, 21 nt, synthetic construct
  source 1..21: mol_type = other RNA; note = The nucleotide modifications are shown in Table 1B
tatttattgacatctacccac

SEQ ID NO: 53 - RNA, 21 nt, synthetic construct
  source 1..21: mol_type = other RNA; note = The nucleotide modifications are shown in Table 1B
tatttattgacatctacccac

SEQ ID NO: 54 - RNA, 21 nt, synthetic construct
  source 1..21: mol_type = other RNA; note = The nucleotide modifications are shown in Table 1B
acatttattgacatctaccca

SEQ ID NO: 55 - RNA, 21 nt, synthetic construct
  source 1..21: mol_type = other RNA; note = The nucleotide modifications are shown in Table 1B
acatttattgacatctaccca

SEQ ID NO: 56 - RNA, 21 nt, synthetic construct
  source 1..21: mol_type = other RNA; note = The nucleotide modifications are shown in Table 1B
taaacattttatttatttgtg

SEQ ID NO: 57 - RNA, 21 nt, synthetic construct
  source 1..21: mol_type = other RNA; note = The nucleotide modifications are shown in Table 1B
taaacattttatttatttgtg

SEQ ID NO: 58 - RNA, 21 nt, synthetic construct
  source 1..21: mol_type = other RNA; note = The nucleotide modifications are shown in Table 1B
atttattgacatctacccact

SEQ ID NO: 59 - RNA, 21 nt, synthetic construct
  source 1..21: mol_type = other RNA; note = The nucleotide modifications are shown in Table 1B
attttttgtttctgagtcata

SEQ ID NO: 60 - RNA, 21 nt, synthetic construct
  source 1..21: mol_type = other RNA; note = The nucleotide modifications are shown in Table 1B
ttctatttctttcttgaatta

SEQ ID NO: 61 - RNA, 19 nt, Homo sapiens
  source 1..19: mol_type = mRNA
caaatcaaccataggtcca

SEQ ID NO: 62 - RNA, 19 nt, Homo sapiens
  source 1..19: mol_type = mRNA
aaccataggtccaagaaca

SEQ ID NO: 63 - RNA, 19 nt, Homo sapiens
  source 1..19: mol_type = mRNA
accataggtccaagaacaa

SEQ ID NO: 64 - RNA, 19 nt, Homo sapiens
  source 1..19: mol_type = mRNA
ccataggtccaagaacaat

SEQ ID NO: 65 - RNA, 19 nt, Homo sapiens
  source 1..19: mol_type = mRNA
cataggtccaagaacaatt

SEQ ID NO: 66 - RNA, 19 nt, Homo sapiens
  source 1..19: mol_type = mRNA
ggtccaagaacaattgtct

SEQ ID NO: 67 - RNA, 19 nt, Homo sapiens
  source 1..19: mol_type = mRNA
gggaggcatgagtgagcta

SEQ ID NO: 68 - RNA, 19 nt, Homo sapiens
  source 1..19: mol_type = mRNA
aggactatctcaagagatt

SEQ ID NO: 69 - RNA, 19 nt, Homo sapiens
  source 1..19: mol_type = mRNA
ggactatctcaagagattt

SEQ ID NO: 70 - RNA, 19 nt, Homo sapiens
  source 1..19: mol_type = mRNA
gactatctcaagagatttt

SEQ ID NO: 71 - RNA, 19 nt, Homo sapiens
  source 1..19: mol_type = mRNA
ctctatgactcagaaacaa

SEQ ID NO: 72 - RNA, 19 nt, Homo sapiens
  source 1..19: mol_type = mRNA
ctatgactcagaaacaaaa

SEQ ID NO: 73 - RNA, 19 nt, Homo sapiens
  source 1..19: mol_type = mRNA
cagaaacaaaaaatgccaa

SEQ ID NO: 74 - RNA, 19 nt, Homo sapiens
  source 1..19: mol_type = mRNA
gaaacaaaaaatgccaaca

SEQ ID NO: 75 - RNA, 19 nt, Homo sapiens
  source 1..19: mol_type = mRNA
caaaaaatgccaacagttt

SEQ ID NO: 76 - RNA, 19 nt, Homo sapiens
  source 1..19: mol_type = mRNA
aaaaaatgccaacagttta

SEQ ID NO: 77 - RNA, 19 nt, Homo sapiens
  source 1..19: mol_type = mRNA
aaatgccaacagtttagaa

SEQ ID NO: 78 - RNA, 19 nt, Homo sapiens
  source 1..19: mol_type = mRNA
gccaacagtttagaagcca

SEQ ID NO: 79 - RNA, 19 nt, Homo sapiens
  source 1..19: mol_type = mRNA
ccaacagtttagaagccaa

SEQ ID NO: 80 - RNA, 19 nt, Homo sapiens
  source 1..19: mol_type = mRNA
agtttagaagccaaactca

SEQ ID NO: 81 - RNA, 19 nt, Homo sapiens
  source 1..19: mol_type = mRNA
gtttagaagccaaactcaa

SEQ ID NO: 82 - RNA, 19 nt, Homo sapiens
  source 1..19: mol_type = mRNA
gaagccaaactcaaggaga

SEQ ID NO: 83 - RNA, 19 nt, Homo sapiens
  source 1..19: mol_type = mRNA
gaaataatgcagaagccca

SEQ ID NO: 84 - RNA, 19 nt, Homo sapiens
  source 1..19: mol_type = mRNA
gcagaagcccagatgtgga

SEQ ID NO: 85 - RNA, 19 nt, Homo sapiens
  source 1..19: mol_type = mRNA
gcccagatgtggagtgcca

SEQ ID NO: 86 - RNA, 19 nt, Homo sapiens
  source 1..19: mol_type = mRNA
aatactcactatttccaaa

SEQ ID NO: 87 - RNA, 19 nt, Homo sapiens
  source 1..19: mol_type = mRNA
tactcactatttccaaata

SEQ ID NO: 88 - RNA, 19 nt, Homo sapiens
  source 1..19: mol_type = mRNA
ctatttccaaatagcccaa

SEQ ID NO: 89 - RNA, 19 nt, Homo sapiens
  source 1..19: mol_type = mRNA
ccaaatagcccaaaatgga

SEQ ID NO: 90 - RNA, 19 nt, Homo sapiens
  source 1..19: mol_type = mRNA
agcccaaaatggacttcca

SEQ ID NO: 91 - RNA, 19 nt, Homo sapiens
  source 1..19: mol_type = mRNA
gcccaaaatggacttccaa

SEQ ID NO: 92 - RNA, 19 nt, Homo sapiens
  source 1..19: mol_type = mRNA
cccaaaatggacttccaaa

SEQ ID NO: 93 - RNA, 19 nt, Homo sapiens
  source 1..19: mol_type = mRNA
atcatatactcgagactta

SEQ ID NO: 94 - RNA, 19 nt, Homo sapiens
  source 1..19: mol_type = mRNA
actcgagacttaccgcata

SEQ ID NO: 95 - RNA, 19 nt, Homo sapiens
  source 1..19: mol_type = mRNA
cgattagtgtcaaaggctt

SEQ ID NO: 96 - RNA, 19 nt, Homo sapiens
  source 1..19: mol_type = mRNA
gattagtgtcaaaggcttt

SEQ ID NO: 97 - RNA, 19 nt, Homo sapiens
  source 1..19: mol_type = mRNA
gtgtcaaaggctttaaaca

SEQ ID NO: 98 - RNA, 19 nt, Homo sapiens
  source 1..19: mol_type = mRNA
tgtcaaaggctttaaacat

SEQ ID NO: 99 - RNA, 19 nt, Homo sapiens
  source 1..19: mol_type = mRNA
gcaaagagatccccctgca

SEQ ID NO: 100 - RNA, 19 nt, Homo sapiens
  source 1..19: mol_type = mRNA
gagatccccctgcatttca

SEQ ID NO: 101 - RNA, 19 nt, Homo sapiens
  source 1..19: mol_type = mRNA
ccccctgcatttcaggaaa

SEQ ID NO: 102 - RNA, 19 nt, Homo sapiens
  source 1..19: mol_type = mRNA
cctgcatttcaggaaagtt

SEQ ID NO: 103 - RNA, 19 nt, Homo sapiens
  source 1..19: mol_type = mRNA
gcatttcaggaaagttgta

SEQ ID NO: 104 - RNA, 19 nt, Homo sapiens
  source 1..19: mol_type = mRNA
caggaaagttgtatgggga

SEQ ID NO: 105 - RNA, 19 nt, Homo sapiens
  source 1..19: mol_type = mRNA
aggaaagttgtatggggaa

SEQ ID NO: 106 - RNA, 19 nt, Homo sapiens
  source 1..19: mol_type = mRNA
ggggaactgctgacatcat

SEQ ID NO: 107 - RNA, 19 nt, Homo sapiens
  source 1..19: mol_type = mRNA
ggaactgctgacatcatga

SEQ ID NO: 108 - RNA, 19 nt, Homo sapiens
  source 1..19: mol_type = mRNA
gaactgctgacatcatgat

SEQ ID NO: 109 - RNA, 19 nt, Homo sapiens
  source 1..19: mol_type = mRNA
ctgacatcatgattggctt

SEQ ID NO: 110 - RNA, 19 nt, Homo sapiens
  source 1..19: mol_type = mRNA
caggaaacacgctggctca

SEQ ID NO: 111 - RNA, 19 nt, Homo sapiens
  source 1..19: mol_type = mRNA
cacgctggctcatgccttt

SEQ ID NO: 112 - RNA, 19 nt, Homo sapiens
  source 1..19: mol_type = mRNA
tcacttcgatgaggatgaa

SEQ ID NO: 113 - RNA, 19 nt, Homo sapiens
  source 1..19: mol_type = mRNA
ggatgaacgctggacggat

SEQ ID NO: 114 - RNA, 19 nt, Homo sapiens
  source 1..19: mol_type = mRNA
gacggatggtagcagtcta

SEQ ID NO: 115 - RNA, 19 nt, Homo sapiens
  source 1..19: mol_type = mRNA
agatccccaaaattttaaa

SEQ ID NO: 116 - RNA, 19 nt, Homo sapiens
  source 1..19: mol_type = mRNA
ccccaaaattttaaacttt

SEQ ID NO: 117 - RNA, 19 nt, Homo sapiens
  source 1..19: mol_type = mRNA
cccaaaattttaaacttta

SEQ ID NO: 118 - RNA, 19 nt, Homo sapiens
  source 1..19: mol_type = mRNA
aaactttcccaggatgata

SEQ ID NO: 119 - RNA, 19 nt, Homo sapiens
  source 1..19: mol_type = mRNA
gatattaaaggcattcaga

SEQ ID NO: 120 - RNA, 19 nt, Homo sapiens
  source 1..19: mol_type = mRNA
atattaaaggcattcagaa

SEQ ID NO: 121 - RNA, 19 nt, Homo sapiens
  source 1..19: mol_type = genomic RNA
tattaaaggcattcagaaa

SEQ ID NO: 122 - RNA, 19 nt, Homo sapiens
  source 1..19: mol_type = mRNA
ttcagaaactatatggaaa

SEQ ID NO: 123 - RNA, 19 nt, Homo sapiens
  source 1..19: mol_type = mRNA
cagaaactatatggaaaga

SEQ ID NO: 124 - RNA, 19 nt, Homo sapiens
  source 1..19: mol_type = mRNA
gaaactatatggaaagaga

SEQ ID NO: 125 - RNA, 19 nt, Homo sapiens
  source 1..19: mol_type = mRNA
aaactatatggaaagagaa

SEQ ID NO: 126 - RNA, 19 nt, Homo sapiens
  source 1..19: mol_type = mRNA
ctatatggaaagagaagta

SEQ ID NO: 127 - RNA, 19 nt, Homo sapiens
  source 1..19: mol_type = mRNA
atatggaaagagaagtaat

SEQ ID NO: 128 - RNA, 19 nt, Homo sapiens
  source 1..19: mol_type = mRNA
tggaaagagaagtaattca

SEQ ID NO: 129 - RNA, 19 nt, Homo sapiens
  source 1..19: mol_type = mRNA
ggaaagagaagtaattcaa

SEQ ID NO: 130 - RNA, 19 nt, Homo sapiens
  source 1..19: mol_type = mRNA
aaagagaagtaattcaaga

SEQ ID NO: 131 - RNA, 19 nt, Homo sapiens
  source 1..19: mol_type = mRNA
aagagaagtaattcaagaa

SEQ ID NO: 132 - RNA, 19 nt, Homo sapiens
  source 1..19: mol_type = mRNA
agagaagtaattcaagaaa

SEQ ID NO: 133 - RNA, 19 nt, Homo sapiens
  source 1..19: mol_type = mRNA
gagaagtaattcaagaaaa

SEQ ID NO: 134 - RNA, 19 nt, Homo sapiens
  source 1..19: mol_type = mRNA
agaagtaattcaagaaaga

SEQ ID NO: 135 - RNA, 19 nt, Homo sapiens
  source 1..19: mol_type = mRNA
gaagtaattcaagaaagaa

SEQ ID NO: 136 - RNA, 19 nt, Homo sapiens
  source 1..19: mol_type = mRNA
aagtaattcaagaaagaaa

SEQ ID NO: 137 - RNA, 19 nt, Homo sapiens
  source 1..19: mol_type = mRNA
gtaattcaagaaagaaata

SEQ ID NO: 138 - RNA, 19 nt, Homo sapiens
  source 1..19: mol_type = mRNA
aattcaagaaagaaataga

SEQ ID NO: 139 - RNA, 19 nt, Homo sapiens
  source 1..19: mol_type = mRNA
caagaaagaaatagaaact

SEQ ID NO: 140 - RNA, 19 nt, Homo sapiens
  source 1..19: mol_type = mRNA
agaaagaaatagaaactta

SEQ ID NO: 141 - RNA, 19 nt, Homo sapiens
  source 1..19: mol_type = mRNA
gaaagaaatagaaacttca

SEQ ID NO: 142 - RNA, 19 nt, Homo sapiens
  source 1..19: mol_type = mRNA
tatcattgttgcacaatca

SEQ ID NO: 143 - RNA, 19 nt, Homo sapiens
  source 1..19: mol_type = mRNA
tcattgttgcacaatcaga

SEQ ID NO: 144 - RNA, 19 nt, Homo sapiens
  source 1..19: mol_type = mRNA
gcaattatgtcaccctttt

SEQ ID NO: 145 - RNA, 19 nt, Homo sapiens
  source 1..19: mol_type = mRNA
gaatgtctttcactccttt

SEQ ID NO: 146 - RNA, 19 nt, Homo sapiens
  source 1..19: mol_type = mRNA
gtagatgtcaataaatgtt

SEQ ID NO: 147 - RNA, 19 nt, Homo sapiens
  source 1..19: mol_type = mRNA
agatgtcaataaatgttaa

SEQ ID NO: 148 - RNA, 19 nt, Homo sapiens
  source 1..19: mol_type = mRNA
cacaaataaataaaatgtt

SEQ ID NO: 149 - RNA, 19 nt, Homo sapiens
  source 1..19: mol_type = mRNA
acaaataaataaaatgttt

SEQ ID NO: 150 - RNA, 19 nt, Homo sapiens
  source 1..19: mol_type = mRNA
aaataaataaaatgtttat

SEQ ID NO: 151 - RNA, 19 nt, Homo sapiens
  source 1..19: mol_type = mRNA
aaataaaatgtttattcca

SEQ ID NO: 152 - RNA, 21 nt, Homo sapiens
  source 1..21: mol_type = mRNA
tggacctatggttgatttggt

SEQ ID NO: 153 - RNA, 21 nt, Homo sapiens
  source 1..21: mol_type = mRNA
tgttcttggacctatggttga

SEQ ID NO: 154 - RNA, 21 nt, Homo sapiens
  source 1..21: mol_type = mRNA
ttgttcttggacctatggttg

SEQ ID NO: 155 - RNA, 21 nt, Homo sapiens
  source 1..21: mol_type = mRNA
attgttcttggacctatggtt

SEQ ID NO: 156 - RNA, 21 nt, Homo sapiens
  source 1..21: mol_type = mRNA
aattgttcttggacctatggt

SEQ ID NO: 157 - RNA, 21 nt, Homo sapiens
  source 1..21: mol_type = mRNA
agacaattgttcttggaccta

SEQ ID NO: 158 - RNA, 21 nt, Homo sapiens
  source 1..21: mol_type = mRNA
tagctcactcatgcctcccgc

SEQ ID NO: 159 - RNA, 21 nt, Homo sapiens
  source 1..21: mol_type = mRNA
aatctcttgagatagtcctga

SEQ ID NO: 160 - RNA, 21 nt, Homo sapiens
  source 1..21: mol_type = mRNA
aaatctcttgagatagtcctg

SEQ ID NO: 161 - RNA, 21 nt, Homo sapiens
  source 1..21: mol_type = mRNA
aaaatctcttgagatagtcct

SEQ ID NO: 162 - RNA, 21 nt, Homo sapiens
  source 1..21: mol_type = mRNA
ttgtttctgagtcatagagat

SEQ ID NO: 163 - RNA, 21 nt, Homo sapiens
  source 1..21: mol_type = mRNA
ttttgtttctgagtcatagag

SEQ ID NO: 164 - RNA, 21 nt, Homo sapiens
  source 1..21: mol_type = mRNA
ttggcattttttgtttctgag

SEQ ID NO: 165 - RNA, 21 nt, Homo sapiens
  source 1..21: mol_type = mRNA
tgttggcattttttgtttctg

SEQ ID NO: 166 - RNA, 21 nt, Homo sapiens
  source 1..21: mol_type = mRNA
aaactgttggcattttttgtt

SEQ ID NO: 167 - RNA, 21 nt, Homo sapiens
  source 1..21: mol_type = mRNA
taaactgttggcattttttgt

SEQ ID NO: 168 - RNA, 21 nt, Homo sapiens
  source 1..21: mol_type = mRNA
ttctaaactgttggcattttt

SEQ ID NO: 169 - RNA, 21 nt, Homo sapiens
  source 1..21: mol_type = mRNA
tggcttctaaactgttggcat

SEQ ID NO: 170 - RNA, 21 nt, Homo sapiens
  source 1..21: mol_type = mRNA
ttggcttctaaactgttggca

SEQ ID NO: 171 - RNA, 21 nt, Homo sapiens
  source 1..21: mol_type = mRNA
tgagtttggcttctaaactgt

SEQ ID NO: 172 - RNA, 21 nt, Homo sapiens
  source 1..21: mol_type = mRNA
ttgagtttggcttctaaactg

SEQ ID NO: 173 - RNA, 21 nt, Homo sapiens
  source 1..21: mol_type = mRNA
tctccttgagtttggcttcta

SEQ ID NO: 174 - RNA, 21 nt, Homo sapiens
  source 1..21: mol_type = mRNA
tgggcttctgcattatttcta

SEQ ID NO: 175 - RNA, 21 nt, Homo sapiens
  source 1..21: mol_type = mRNA
tccacatctgggcttctgcat

SEQ ID NO: 176 - RNA, 21 nt, Homo sapiens
  source 1..21: mol_type = mRNA
tggcactccacatctgggctt

SEQ ID NO: 177 - RNA, 21 nt, Homo sapiens
  source 1..21: mol_type = mRNA
tttggaaatagtgagtattct

SEQ ID NO: 178 - RNA, 21 nt, Homo sapiens
  source 1..21: mol_type = mRNA
tatttggaaatagtgagtatt

SEQ ID NO: 179 - RNA, 21 nt, Homo sapiens
  source 1..21: mol_type = mRNA
ttgggctatttggaaatagtg

SEQ ID NO: 180 - RNA, 21 nt, Homo sapiens
  source 1..21: mol_type = mRNA
tccattttgggctatttggaa

SEQ ID NO: 181 - RNA, 21 nt, Homo sapiens
  source 1..21: mol_type = mRNA
tggaagtccattttgggctat

SEQ ID NO: 182 - RNA, 21 nt, Homo sapiens
  source 1..21: mol_type = mRNA
ttggaagtccattttgggcta

SEQ ID NO: 183 - RNA, 21 nt, Homo sapiens
  source 1..21: mol_type = mRNA
tttggaagtccattttgggct

SEQ ID NO: 184 - RNA, 21 nt, Homo sapiens
  source 1..21: mol_type = mRNA
taagtctcgagtatatgatac

SEQ ID NO: 185 - RNA, 21 nt, Homo sapiens
  source 1..21: mol_type = mRNA
tatgcggtaagtctcgagtat

SEQ ID NO: 186 - RNA, 21 nt, Homo sapiens
  source 1..21: mol_type = mRNA
aagcctttgacactaatcgat

SEQ ID NO: 187 - RNA, 21 nt, Homo sapiens
  source 1..21: mol_type = mRNA
aaagcctttgacactaatcga

SEQ ID NO: 188 - RNA, 21 nt, Homo sapiens
  source 1..21: mol_type = mRNA
tgtttaaagcctttgacacta

SEQ ID NO: 189 - RNA, 21 nt, Homo sapiens
  source 1..21: mol_type = mRNA
atgtttaaagcctttgacact

SEQ ID NO: 190 - RNA, 21 nt, Homo sapiens
  source 1..21: mol_type = mRNA
tgcagggggatctctttgccc

SEQ ID NO: 191 - RNA, 21 nt, Homo sapiens
  source 1..21: mol_type = mRNA
tgaaatgcagggggatctctt

SEQ ID NO: 192 - RNA, 21 nt, Homo sapiens
  source 1..21: mol_type = mRNA
tttcctgaaatgcagggggat

SEQ ID NO: 193 - RNA, 21 nt, Homo sapiens
  source 1..21: mol_type = mRNA
aactttcctgaaatgcagggg

SEQ ID NO: 194 - RNA, 21 nt, Homo sapiens
  source 1..21: mol_type = mRNA
tacaactttcctgaaatgcag

SEQ ID NO: 195 - RNA, 21 nt, Homo sapiens
  source 1..21: mol_type = mRNA
tccccatacaactttcctgaa

SEQ ID NO: 196 - RNA, 21 nt, Homo sapiens
  source 1..21: mol_type = mRNA
ttccccatacaactttcctga

SEQ ID NO: 197 - RNA, 21 nt, Homo sapiens
  source 1..21: mol_type = mRNA
atgatgtcagcagttccccat

SEQ ID NO: 198 - RNA, 21 nt, Homo sapiens
  source 1..21: mol_type = mRNA
tcatgatgtcagcagttcccc

SEQ ID NO: 199 - RNA, 21 nt, Homo sapiens
  source 1..21: mol_type = mRNA
atcatgatgtcagcagttccc

SEQ ID NO: 200 - RNA, 21 nt, Homo sapiens
  source 1..21: mol_type = mRNA
aagccaatcatgatgtcagca

SEQ ID NO: 201 - RNA, 21 nt, Homo sapiens
  source 1..21: mol_type = mRNA
tgagccagcgtgtttcctggc

SEQ ID NO: 202 - RNA, 21 nt, Homo sapiens
  source 1..21: mol_type = mRNA
aaaggcatgagccagcgtgtt

SEQ ID NO: 203 - RNA, 21 nt, Homo sapiens
  source 1..21: mol_type = mRNA
ttcatcctcatcgaagtgagc

SEQ ID NO: 204 - RNA, 21 nt, Homo sapiens
  source 1..21: mol_type = mRNA
atccgtccagcgttcatcctc

SEQ ID NO: 205 - RNA, 21 nt, Homo sapiens
  source 1..21: mol_type = mRNA
tagactgctaccatccgtcca

SEQ ID NO: 206 - RNA, 21 nt, Homo sapiens
  source 1..21: mol_type = mRNA
tttaaaattttggggatctcc

SEQ ID NO: 207 - RNA, 21 nt, Homo sapiens
  source 1..21: mol_type = mRNA
aaagtttaaaattttggggat

SEQ ID NO: 208 - RNA, 21 nt, Homo sapiens
  source 1..21: mol_type = mRNA
taaagtttaaaattttgggga

SEQ ID NO: 209 - RNA, 21 nt, Homo sapiens
  source 1..21: mol_type = mRNA
tatcatcctgggaaagtttaa

SEQ ID NO: 210 - RNA, 21 nt, Homo sapiens
  source 1..21: mol_type = mRNA
tctgaatgcctttaatatcat

SEQ ID NO: 211 - RNA, 21 nt, Homo sapiens
  source 1..21: mol_type = mRNA
ttctgaatgcctttaatatca

SEQ ID NO: 212 - RNA, 21 nt, Homo sapiens
  source 1..21: mol_type = mRNA
tttctgaatgcctttaatatc

SEQ ID NO: 213 - RNA, 21 nt, Homo sapiens
  source 1..21: mol_type = mRNA
tttccatatagtttctgaatg

SEQ ID NO: 214 - RNA, 21 nt, Homo sapiens
  source 1..21: mol_type = mRNA
tctttccatatagtttctgaa

SEQ ID NO: 215 - RNA, 21 nt, Homo sapiens
  source 1..21: mol_type = mRNA
tctctttccatatagtttctg

SEQ ID NO: 216 - RNA, 21 nt, Homo sapiens
  source 1..21: mol_type = mRNA
ttctctttccatatagtttct

SEQ ID NO: 217 - RNA, 21 nt, Homo sapiens
  source 1..21: mol_type = mRNA
tacttctctttccatatagtt

SEQ ID NO: 218 - RNA, 21 nt, Homo sapiens
  source 1..21: mol_type = mRNA
attacttctctttccatatag

SEQ ID NO: 219 - RNA, 21 nt, Homo sapiens
  source 1..21: mol_type = mRNA
tgaattacttctctttccata

SEQ ID NO: 220 - RNA, 21 nt, Homo sapiens
  source 1..21: mol_type = mRNA
ttgaattacttctctttccat

SEQ ID NO: 221 - RNA, 21 nt, Homo sapiens
  source 1..21: mol_type = mRNA
tcttgaattacttctctttcc

SEQ ID NO: 222 - RNA, 21 nt, Homo sapiens
  source 1..21: mol_type = mRNA
ttcttgaattacttctctttc

SEQ ID NO: 223 - RNA, 21 nt, Homo sapiens
  source 1..21: mol_type = mRNA
tttcttgaattacttctcttt

SEQ ID NO: 224 - RNA, 21 nt, Homo sapiens
  source 1..21: mol_type = mRNA
ttttcttgaattacttctctt

SEQ ID NO: 225 - RNA, 21 nt, Homo sapiens
  source 1..21: mol_type = mRNA
tctttcttgaattacttctct

SEQ ID NO: 226 - RNA, 21 nt, Homo sapiens
  source 1..21: mol_type = mRNA
ttctttcttgaattacttctc

SEQ ID NO: 227 - RNA, 21 nt, Homo sapiens
  source 1..21: mol_type = mRNA
tttctttcttgaattacttct

SEQ ID NO: 228 - RNA, 21 nt, Homo sapiens
  source 1..21: mol_type = mRNA
tatttctttcttgaattactt

SEQ ID NO: 229 - RNA, 21 nt, Homo sapiens
  source 1..21: mol_type = mRNA
tctatttctttcttgaattac

SEQ ID NO: 230 - RNA, 21 nt, Homo sapiens
  source 1..21: mol_type = mRNA
agtttctatttctttcttgaa

SEQ ID NO: 231 - RNA, 21 nt, Homo sapiens
  source 1..21: mol_type = mRNA
taagtttctatttctttcttg

SEQ ID NO: 232 - RNA, 21 nt, Homo sapiens
  source 1..21: mol_type = mRNA
tgaagtttctatttctttctt

SEQ ID NO: 233 - RNA, 21 nt, Homo sapiens
  source 1..21: mol_type = mRNA
tgattgtgcaacaatgatata

SEQ ID NO: 234 - RNA, 21 nt, Homo sapiens
  source 1..21: mol_type = mRNA
tctgattgtgcaacaatgata

SEQ ID NO: 235 - RNA, 21 nt, Homo sapiens
  source 1..21: mol_type = mRNA
aaaagggtgacataattgcta

SEQ ID NO: 236 - RNA, 21 nt, Homo sapiens
  source 1..21: mol_type = mRNA
aaaggagtgaaagacattcaa

SEQ ID NO: 237 - RNA, 21 nt, Homo sapiens
  source 1..21: mol_type = mRNA
aacatttattgacatctaccc

SEQ ID NO: 238 - RNA, 21 nt, Homo sapiens
  source 1..21: mol_type = mRNA
ttaacatttattgacatctac

SEQ ID NO: 239 - RNA, 21 nt, Homo sapiens
  source 1..21: mol_type = mRNA
aacattttatttatttgtgta

SEQ ID NO: 240 - RNA, 21 nt, Homo sapiens
  source 1..21: mol_type = mRNA
aaacattttatttatttgtgt

SEQ ID NO: 241 - RNA, 21 nt, Homo sapiens
  source 1..21: mol_type = mRNA
ataaacattttatttatttgt

SEQ ID NO: 242 - RNA, 21 nt, Homo sapiens
  source 1..21: mol_type = mRNA
tggaataaacattttatttat

SEQ ID NO: 243 - RNA, 19 nt, synthetic construct
  source 1..19: mol_type = other RNA; note = The nucleotide modifications are shown in Table 1B
caaatcaaccataggtcca

SEQ ID NO: 244 - RNA, 19 nt, synthetic construct
  source 1..19: mol_type = other RNA; note = The nucleotide modifications are shown in Table 1B
aaccataggtccaagaaca

SEQ ID NO: 245 - RNA, 19 nt, synthetic construct
  source 1..19: mol_type = other RNA; note = The nucleotide modifications are shown in Table 1B
accataggtccaagaacaa

SEQ ID NO: 246 - RNA, 19 nt, synthetic construct
  source 1..19: mol_type = other RNA; note = The nucleotide modifications are shown in Table 1B
ccataggtccaagaacaat

SEQ ID NO: 247 - RNA, 19 nt, synthetic construct
  source 1..19: mol_type = other RNA; note = The nucleotide modifications are shown in Table 1B
cataggtccaagaacaatt

SEQ ID NO: 248 - RNA, 19 nt, synthetic construct
  source 1..19: mol_type = other RNA; note = The nucleotide modifications are shown in Table 1B
ggtccaagaacaattgtct

SEQ ID NO: 249 - RNA, 19 nt, synthetic construct
  source 1..19: mol_type = other RNA; note = The nucleotide modifications are shown in Table 1B
gggaggcatgagtgagcta

SEQ ID NO: 250 - RNA, 19 nt, synthetic construct
  source 1..19: mol_type = other RNA; note = The nucleotide modifications are shown in Table 1B
aggactatctcaagagatt

SEQ ID NO: 251 - RNA, 19 nt, synthetic construct
  source 1..19: mol_type = other RNA; note = The nucleotide modifications are shown in Table 1B
ggactatctcaagagattt

SEQ ID NO: 252 - RNA, 19 nt, synthetic construct
  source 1..19: mol_type = other RNA; note = The nucleotide modifications are shown in Table 1B
gactatctcaagagatttt

SEQ ID NO: 253 - RNA, 19 nt, synthetic construct
  source 1..19: mol_type = other RNA; note = The nucleotide modifications are shown in Table 1B
ctctatgactcagaaacaa

SEQ ID NO: 254 - RNA, 19 nt, synthetic construct
  source 1..19: mol_type = other RNA; note = The nucleotide modifications are shown in Table 1B
ctatgactcagaaacaaaa

SEQ ID NO: 255 - RNA, 19 nt, synthetic construct
  source 1..19: mol_type = other RNA; note = The nucleotide modifications are shown in Table 1B
cagaaacaaaaaatgccaa

SEQ ID NO: 256 - RNA, 19 nt, synthetic construct
  source 1..19: mol_type = other RNA; note = The nucleotide modifications are shown in Table 1B
gaaacaaaaaatgccaaca

SEQ ID NO: 257 - RNA, 19 nt, synthetic construct
  source 1..19: mol_type = other RNA; note = The nucleotide modifications are shown in Table 1B
caaaaaatgccaacagttt

SEQ ID NO: 258 - RNA, 19 nt, synthetic construct
  source 1..19: mol_type = other RNA; note = The nucleotide modifications are shown in Table 1B
aaaaaatgccaacagttta

SEQ ID NO: 259 - RNA, 19 nt, synthetic construct
  source 1..19: mol_type = other RNA; note = The nucleotide modifications are shown in Table 1B
aaatgccaacagtttagaa

SEQ ID NO: 260 - RNA, 19 nt, synthetic construct
  source 1..19: mol_type = other RNA; note = The nucleotide modifications are shown in Table 1B
gccaacagtttagaagcca

SEQ ID NO: 261 - RNA, 19 nt, synthetic construct
  source 1..19: mol_type = other RNA; note = The nucleotide modifications are shown in Table 1B
ccaacagtttagaagccaa

SEQ ID NO: 262 - RNA, 19 nt, synthetic construct
  source 1..19: mol_type = other RNA; note = The nucleotide modifications are shown in Table 1B
agtttagaagccaaactca

SEQ ID NO: 263 - RNA, 19 nt, synthetic construct
  source 1..19: mol_type = other RNA; note = The nucleotide modifications are shown in Table 1B
gtttagaagccaaactcaa

SEQ ID NO: 264 - RNA, 19 nt, synthetic construct
  source 1..19: mol_type = other RNA; note = The nucleotide modifications are shown in Table 1B
gaagccaaactcaaggaga

SEQ ID NO: 265 - RNA, 19 nt, synthetic construct
  source 1..19: mol_type = other RNA; note = The nucleotide modifications are shown in Table 1B
gaaataatgcagaagccca

SEQ ID NO: 266 - RNA, 19 nt, synthetic construct
  source 1..19: mol_type = other RNA; note = The nucleotide modifications are shown in Table 1B
gcagaagcccagatgtgga

SEQ ID NO: 267 - RNA, 19 nt, synthetic construct
  source 1..19: mol_type = other RNA; note = The nucleotide modifications are shown in Table 1B
gcccagatgtggagtgcca

SEQ ID NO: 268 - RNA, 19 nt, synthetic construct
  source 1..19: mol_type = other RNA; note = The nucleotide modifications are shown in Table 1B
aatactcactatttccaaa

SEQ ID NO: 269 - RNA, 19 nt, synthetic construct
  source 1..19: mol_type = other RNA; note = The nucleotide modifications are shown in Table 1B
tactcactatttccaaata

SEQ ID NO: 270 - RNA, 19 nt, synthetic construct
  source 1..19: mol_type = other RNA; note = The nucleotide modifications are shown in Table 1B
ctatttccaaatagcccaa

SEQ ID NO: 271 - RNA, 19 nt, synthetic construct
  source 1..19: mol_type = other RNA; note = The nucleotide modifications are shown in Table 1B
ccaaatagcccaaaatgga

SEQ ID NO: 272 - RNA, 19 nt, synthetic construct
  source 1..19: mol_type = other RNA; note = The nucleotide modifications are shown in Table 1B
agcccaaaatggacttcca

SEQ ID NO: 273 - RNA, 19 nt, synthetic construct
  source 1..19: mol_type = other RNA; note = The nucleotide modifications are shown in Table 1B
gcccaaaatggacttccaa

SEQ ID NO: 274 - RNA, 19 nt, synthetic construct
  source 1..19: mol_type = other RNA; note = The nucleotide modifications are shown in Table 1B
cccaaaatggacttccaaa

SEQ ID NO: 275 - RNA, 19 nt, synthetic construct
  source 1..19: mol_type = other RNA; note = The nucleotide modifications are shown in Table 1B
atcatatactcgagactta

SEQ ID NO: 276 - RNA, 19 nt, synthetic construct
  source 1..19: mol_type = other RNA; note = The nucleotide modifications are shown in Table 1B
actcgagacttaccgcata

SEQ ID NO: 277 - RNA, 19 nt, synthetic construct
  source 1..19: mol_type = other RNA; note = The nucleotide modifications are shown in Table 1B
cgattagtgtcaaaggctt

SEQ ID NO: 278 - RNA, 19 nt, synthetic construct
  source 1..19: mol_type = other RNA; note = The nucleotide modifications are shown in Table 1B
gattagtgtcaaaggcttt

SEQ ID NO: 279 - RNA, 19 nt, synthetic construct
  source 1..19: mol_type = other RNA; note = The nucleotide modifications are shown in Table 1B
gtgtcaaaggctttaaaca

SEQ ID NO: 280 - RNA, 19 nt, synthetic construct
  source 1..19: mol_type = other RNA; note = The nucleotide modifications are shown in Table 1B
tgtcaaaggctttaaacat

SEQ ID NO: 281 - RNA, 19 nt, synthetic construct
  source 1..19: mol_type = other RNA; note = The nucleotide modifications are shown in Table 1B
gcaaagagatccccctgca

SEQ ID NO: 282 - RNA, 19 nt, synthetic construct
  source 1..19: mol_type = other RNA; note = The nucleotide modifications are shown in Table 1B
gagatccccctgcatttca

SEQ ID NO: 283 - RNA, 19 nt, synthetic construct
  source 1..19: mol_type = other RNA; note = The nucleotide modifications are shown in Table 1B
ccccctgcatttcaggaaa

SEQ ID NO: 284 - RNA, 19 nt, synthetic construct
  source 1..19: mol_type = other RNA; note = The nucleotide modifications are shown in Table 1B
cctgcatttcaggaaagtt

SEQ ID NO: 285 - RNA, 19 nt, synthetic construct
  source 1..19: mol_type = other RNA; note = The nucleotide modifications are shown in Table 1B
gcatttcaggaaagttgta

SEQ ID NO: 286 - RNA, 19 nt, synthetic construct
  source 1..19: mol_type = other RNA; note = The nucleotide modifications are shown in Table 1B
caggaaagttgtatgggga

SEQ ID NO: 287 - RNA, 19 nt, synthetic construct
  source 1..19: mol_type = other RNA; note = The nucleotide modifications are shown in Table 1B
aggaaagttgtatggggaa

SEQ ID NO: 288 - RNA, 19 nt, synthetic construct
  source 1..19: mol_type = other RNA; note = The nucleotide modifications are shown in Table 1B
ggggaactgctgacatcat

SEQ ID NO: 289 - RNA, 19 nt, synthetic construct
  source 1..19: mol_type = other RNA; note = The nucleotide modifications are shown in Table 1B
ggaactgctgacatcatga

SEQ ID NO: 290 - RNA, 19 nt, synthetic construct
  source 1..19: mol_type = other RNA; note = The nucleotide modifications are shown in Table 1B
gaactgctgacatcatgat

SEQ ID NO: 291 - RNA, 19 nt, synthetic construct
  source 1..19: mol_type = other RNA; note = The nucleotide modifications are shown in Table 1B
ctgacatcatgattggctt

SEQ ID NO: 292 - RNA, 19 nt, synthetic construct
  source 1..19: mol_type = other RNA; note = The nucleotide modifications are shown in Table 1B
caggaaacacgctggctca

SEQ ID NO: 293 - RNA, 19 nt, synthetic construct
  source 1..19: mol_type = other RNA; note = The nucleotide modifications are shown in Table 1B
cacgctggctcatgccttt

SEQ ID NO: 294 - RNA, 19 nt, synthetic construct
  source 1..19: mol_type = other RNA; note = The nucleotide modifications are shown in Table 1B
tcacttcgatgaggatgaa

SEQ ID NO: 295 - RNA, 19 nt, synthetic construct
  source 1..19: mol_type = other RNA; note = The nucleotide modifications are shown in Table 1B
ggatgaacgctggacggat

SEQ ID NO: 296 - RNA, 19 nt, synthetic construct
  source 1..19: mol_type = other RNA; note = The nucleotide modifications are shown in Table 1B
gacggatggtagcagtcta

SEQ ID NO: 297 - RNA, 19 nt, synthetic construct
  source 1..19: mol_type = other RNA; note = The nucleotide modifications are shown in Table 1B
agatccccaaaattttaaa

SEQ ID NO: 298 - RNA, 19 nt, synthetic construct
  source 1..19: mol_type = other RNA; note = The nucleotide modifications are shown in Table 1B
ccccaaaattttaaacttt

SEQ ID NO: 299 - RNA, 19 nt, synthetic construct
  source 1..19: mol_type = other RNA; note = The nucleotide modifications are shown in Table 1B
cccaaaattttaaacttta

SEQ ID NO: 300 - RNA, 19 nt, synthetic construct
  source 1..19: mol_type = other RNA; note = The nucleotide modifications are shown in Table 1B
aaactttcccaggatgata

SEQ ID NO: 301 - RNA, 19 nt, synthetic construct
  source 1..19: mol_type = other RNA; note = The nucleotide modifications are shown in Table 1B
gatattaaaggcattcaga

SEQ ID NO: 302 - RNA, 19 nt, synthetic construct
  source 1..19: mol_type = other RNA; note = The nucleotide modifications are shown in Table 1B
atattaaaggcattcagaa

SEQ ID NO: 303 - RNA, 19 nt, synthetic construct
  source 1..19: mol_type = other RNA; note = The nucleotide modifications are shown in Table 1B
tattaaaggcattcagaaa

SEQ ID NO: 304 - RNA, 19 nt, synthetic construct
  source 1..19: mol_type = other RNA; note = The nucleotide modifications are shown in Table 1B
ttcagaaactatatggaaa

SEQ ID NO: 305 - RNA, 19 nt, synthetic construct
  source 1..19: mol_type = other RNA; note = The nucleotide modifications are shown in Table 1B
cagaaactatatggaaaga

SEQ ID NO: 306 - RNA, 19 nt, synthetic construct
  source 1..19: mol_type = other RNA; note = The nucleotide modifications are shown in Table 1B
gaaactatatggaaagaga

SEQ ID NO: 307 - RNA, 19 nt, synthetic construct
  source 1..19: mol_type = other RNA; note = The nucleotide modifications are shown in Table 1B
aaactatatggaaagagaa

SEQ ID NO: 308 - RNA, 19 nt, synthetic construct
  source 1..19: mol_type = other RNA; note = The nucleotide modifications are shown in Table 1B
ctatatggaaagagaagta

SEQ ID NO: 309 - RNA, 19 nt, synthetic construct
  source 1..19: mol_type = other RNA; note = The nucleotide modifications are shown in Table 1B
atatggaaagagaagtaat

SEQ ID NO: 310 - RNA, 19 nt, synthetic construct
  source 1..19: mol_type = other RNA; note = The nucleotide modifications are shown in Table 1B
tggaaagagaagtaattca

SEQ ID NO: 311 - RNA, 19 nt, synthetic construct
  source 1..19: mol_type = other RNA; note = The nucleotide modifications are shown in Table 1B
ggaaagagaagtaattcaa

SEQ ID NO: 312 - RNA, 19 nt, synthetic construct
  source 1..19: mol_type = other RNA; note = The nucleotide modifications are shown in Table 1B
aaagagaagtaattcaaga

SEQ ID NO: 313 - RNA, 19 nt, synthetic construct
  source 1..19: mol_type = other RNA; note = The nucleotide modifications are shown in Table 1B
aagagaagtaattcaagaa

SEQ ID NO: 314 - RNA, 19 nt, synthetic construct
  source 1..19: mol_type = other RNA; note = The nucleotide modifications are shown in Table 1B
agagaagtaattcaagaaa

SEQ ID NO: 315 - RNA, 19 nt, synthetic construct
  source 1..19: mol_type = other RNA; note = The nucleotide modifications are shown in Table 1B
gagaagtaattcaagaaaa

SEQ ID NO: 316 - RNA, 19 nt, synthetic construct
  source 1..19: mol_type = other RNA; note = The nucleotide modifications are shown in Table 1B
agaagtaattcaagaaaga

SEQ ID NO: 317 - RNA, 19 nt, synthetic construct
  source 1..19: mol_type = other RNA; note = The nucleotide modifications are shown in Table 1B
gaagtaattcaagaaagaa

SEQ ID NO: 318 - RNA, 19 nt, synthetic construct
  source 1..19: mol_type = other RNA; note = The nucleotide modifications are shown in Table 1B
aagtaattcaagaaagaaa

SEQ ID NO: 319 - RNA, 19 nt, synthetic construct
  source 1..19: mol_type = other RNA; note = The nucleotide modifications are shown in Table 1B
gtaattcaagaaagaaata

SEQ ID NO: 320 - RNA, 19 nt, synthetic construct
  source 1..19: mol_type = other RNA; note = The nucleotide modifications are shown in Table 1B
aattcaagaaagaaataga

SEQ ID NO: 321 - RNA, 19 nt, synthetic construct
  source 1..19: mol_type = other RNA; note = The nucleotide modifications are shown in Table 1B
caagaaagaaatagaaact

SEQ ID NO: 322 - RNA, 19 nt, synthetic construct
  source 1..19: mol_type = other RNA; note = The nucleotide modifications are shown in Table 1B
agaaagaaatagaaactta

SEQ ID NO: 323 - RNA, 19 nt, synthetic construct
  source 1..19: mol_type = other RNA; note = The nucleotide modifications are shown in Table 1B
gaaagaaatagaaacttca

SEQ ID NO: 324 - RNA, 19 nt, synthetic construct
  source 1..19: mol_type = other RNA; note = The nucleotide modifications are shown in Table 1B
tatcattgttgcacaatca

SEQ ID NO: 325 - RNA, 19 nt, synthetic construct
  source 1..19: mol_type = other RNA; note = The nucleotide modifications are shown in Table 1B
tcattgttgcacaatcaga

SEQ ID NO: 326 - RNA, 19 nt, synthetic construct
  source 1..19: mol_type = other RNA; note = The nucleotide modifications are shown in Table 1B
gcaattatgtcaccctttt

SEQ ID NO: 327 - RNA, 19 nt, synthetic construct
  source 1..19: mol_type = other RNA; note = The nucleotide modifications are shown in Table 1B
gaatgtctttcactccttt

SEQ ID NO: 328 - RNA, 19 nt, synthetic construct
  source 1..19: mol_type = other RNA; note = The nucleotide modifications are shown in Table 1B
gtagatgtcaataaatgtt

SEQ ID NO: 329 - RNA, 19 nt, synthetic construct
  source 1..19: mol_type = other RNA; note = The nucleotide modifications are shown in Table 1B
agatgtcaataaatgttaa

SEQ ID NO: 330 - RNA, 19 nt, synthetic construct
  source 1..19: mol_type = other RNA; note = The nucleotide modifications are shown in Table 1B
cacaaataaataaaatgtt

SEQ ID NO: 331 - RNA, 19 nt, synthetic construct
  source 1..19: mol_type = other RNA; note = The nucleotide modifications are shown in Table 1B
acaaataaataaaatgttt

SEQ ID NO: 332 - RNA, 19 nt, synthetic construct
  source 1..19: mol_type = other RNA; note = The nucleotide modifications are shown in Table 1B
aaataaataaaatgtttat

SEQ ID NO: 333 - RNA, 19 nt, synthetic construct
  source 1..19: mol_type = other RNA; note = The nucleotide modifications are shown in Table 1B
aaataaaatgtttattcca

SEQ ID NO: 334 - RNA, 21 nt, synthetic construct
  source 1..21: mol_type = other RNA; note = The nucleotide modifications are shown in Table 1B
tggacctatggttgatttggt

SEQ ID NO: 335 - RNA, 21 nt, synthetic construct
  source 1..21: mol_type = other RNA; note = The nucleotide modifications are shown in Table 1B
tgttcttggacctatggttga

SEQ ID NO: 336 - RNA, 21 nt, synthetic construct
  source 1..21: mol_type = other RNA; note = The nucleotide modifications are shown in Table 1B
ttgttcttggacctatggttg

SEQ ID NO: 337 - RNA, 21 nt, synthetic construct
  source 1..21: mol_type = other RNA; note = The nucleotide modifications are shown in Table 1B
attgttcttggacctatggtt

SEQ ID NO: 338 - RNA, 21 nt, synthetic construct
  source 1..21: mol_type = other RNA; note = The nucleotide modifications are shown in Table 1B
aattgttcttggacctatggt

SEQ ID NO: 339 - RNA, 21 nt, synthetic construct
  source 1..21: mol_type = other RNA; note = The nucleotide modifications are shown in Table 1B
agacaattgttcttggaccta

SEQ ID NO: 340 - RNA, 21 nt, synthetic construct
  source 1..21: mol_type = other RNA; note = The nucleotide modifications are shown in Table 1B
tagctcactcatgcctcccgc

SEQ ID NO: 341 - RNA, 21 nt, synthetic construct
  source 1..21: mol_type = other RNA; note = The nucleotide modifications are shown in Table 1B
aatctcttgagatagtcctga

SEQ ID NO: 342 - RNA, 21 nt, synthetic construct
  source 1..21: mol_type = other RNA; note = The nucleotide modifications are shown in Table 1B
aaatctcttgagatagtcctg

SEQ ID NO: 343 - RNA, 21 nt, synthetic construct
  source 1..21: mol_type = other RNA; note = The nucleotide modifications are shown in Table 1B
aaaatctcttgagatagtcct

SEQ ID NO: 344 - RNA, 21 nt, synthetic construct
  source 1..21: mol_type = other RNA; note = The nucleotide modifications are shown in Table 1B
ttgtttctgagtcatagagat

SEQ ID NO: 345 - RNA, 21 nt, synthetic construct
  source 1..21: mol_type = other RNA; note = The nucleotide modifications are shown in Table 1B
ttttgtttctgagtcatagag

SEQ ID NO: 346 - RNA, 21 nt, synthetic construct
  source 1..21: mol_type = other RNA; note = The nucleotide modifications are shown in Table 1B
ttggcattttttgtttctgag

SEQ ID NO: 347 - RNA, 21 nt, synthetic construct
  source 1..21: mol_type = other RNA; note = The nucleotide modifications are shown in Table 1B
tgttggcattttttgtttctg

SEQ ID NO: 348 - RNA, 21 nt, synthetic construct
  source 1..21: mol_type = other RNA; note = The nucleotide modifications are shown in Table 1B
aaactgttggcattttttgtt

SEQ ID NO: 349 - RNA, 21 nt, synthetic construct
  source 1..21: mol_type = other RNA; note = The nucleotide modifications are shown in Table 1B
taaactgttggcattttttgt

SEQ ID NO: 350 - RNA, 21 nt, synthetic construct
  source 1..21: mol_type = other RNA; note = The nucleotide modifications are shown in Table 1B
ttctaaactgttggcattttt

SEQ ID NO: 351 - RNA, 21 nt, synthetic construct
  source 1..21: mol_type = other RNA; note = The nucleotide modifications are shown in Table 1B
tggcttctaaactgttggcat

SEQ ID NO: 352 - RNA, 21 nt, synthetic construct
  source 1..21: mol_type = other RNA; note = The nucleotide modifications are shown in Table 1B
ttggcttctaaactgttggca

SEQ ID NO: 353 - RNA, 21 nt, synthetic construct
  source 1..21: mol_type = other RNA; note = The nucleotide modifications are shown in Table 1B
tgagtttggcttctaaactgt

SEQ ID NO: 354 - RNA, 21 nt, synthetic construct
  source 1..21: mol_type = other RNA; note = The nucleotide modifications are shown in Table 1B
ttgagtttggcttctaaactg

SEQ ID NO: 355 - RNA, 21 nt, synthetic construct
  source 1..21: mol_type = other RNA; note = The nucleotide modifications are shown in Table 1B
tctccttgagtttggcttcta

SEQ ID NO: 356 - RNA, 21 nt, synthetic construct
  source 1..21: mol_type = other RNA; note = The nucleotide modifications are shown in Table 1B
tgggcttctgcattatttcta

SEQ ID NO: 357 - RNA, 21 nt, synthetic construct
  source 1..21: mol_type = other RNA; note = The nucleotide modifications are shown in Table 1B
tccacatctgggcttctgcat

SEQ ID NO: 358 - RNA, 21 nt, synthetic construct
  source 1..21: mol_type = other RNA; note = The nucleotide modifications are shown in Table 1B
tggcactccacatctgggctt

SEQ ID NO: 359 - RNA, 21 nt, synthetic construct
  source 1..21: mol_type = other RNA; note = The nucleotide modifications are shown in Table 1B
tttggaaatagtgagtattct

SEQ ID NO: 360 - RNA, 21 nt, synthetic construct
  source 1..21: mol_type = other RNA; note = The nucleotide modifications are shown in Table 1B
tatttggaaatagtgagtatt

SEQ ID NO: 361 - RNA, 21 nt, synthetic construct
  source 1..21: mol_type = other RNA; note = The nucleotide modifications are shown in Table 1B
ttgggctatttggaaatagtg

SEQ ID NO: 362 - RNA, 21 nt, synthetic construct
  source 1..21: mol_type = other RNA; note = The nucleotide modifications are shown in Table 1B
tccattttgggctatttggaa

SEQ ID NO: 363 - RNA, 21 nt, synthetic construct
  source 1..21: mol_type = other RNA; note = The nucleotide modifications are shown in Table 1B
tggaagtccattttgggctat

SEQ ID NO: 364 - RNA, 21 nt, synthetic construct
  source 1..21: mol_type = other RNA; note = The nucleotide modifications are shown in Table 1B
ttggaagtccattttgggcta

SEQ ID NO: 365 - RNA, 21 nt, synthetic construct
  source 1..21: mol_type = other RNA; note = The nucleotide modifications are shown in Table 1B
tttggaagtccattttgggct

SEQ ID NO: 366 - RNA, 21 nt, synthetic construct
  source 1..21: mol_type = other RNA; note = The nucleotide modifications are shown in Table 1B
taagtctcgagtatatgatac

SEQ ID NO: 367 - RNA, 21 nt, synthetic construct
  source 1..21: mol_type = other RNA; note = The nucleotide modifications are shown in Table 1B
tatgcggtaagtctcgagtat

SEQ ID NO: 368 - RNA, 21 nt, synthetic construct
  source 1..21: mol_type = other RNA; note = The nucleotide modifications are shown in Table 1B
aagcctttgacactaatcgat

SEQ ID NO: 369 - RNA, 21 nt, synthetic construct
  source 1..21: mol_type = other RNA; note = The nucleotide modifications are shown in Table 1B
aaagcctttgacactaatcga

SEQ ID NO: 370 - RNA, 21 nt, synthetic construct
  source 1..21: mol_type = other RNA; note = The nucleotide modifications are shown in Table 1B
tgtttaaagcctttgacacta

SEQ ID NO: 371 - RNA, 21 nt, synthetic construct
  source 1..21: mol_type = other RNA; note = The nucleotide modifications are shown in Table 1B
atgtttaaagcctttgacact

SEQ ID NO: 372 - RNA, 21 nt, synthetic construct
  source 1..21: mol_type = other RNA; note = The nucleotide modifications are shown in Table 1B
tgcagggggatctctttgccc

SEQ ID NO: 373 - RNA, 21 nt, synthetic construct
  source 1..21: mol_type = other RNA; note = The nucleotide modifications are shown in Table 1B
tgaaatgcagggggatctctt

SEQ ID NO: 374 - RNA, 21 nt, synthetic construct
  source 1..21: mol_type = other RNA; note = The nucleotide modifications are shown in Table 1B
tttcctgaaatgcagggggat

SEQ ID NO: 375 - RNA, 21 nt, synthetic construct
  source 1..21: mol_type = other RNA; note = The nucleotide modifications are shown in Table 1B
aactttcctgaaatgcagggg

SEQ ID NO: 376 - RNA, 21 nt, synthetic construct
  source 1..21: mol_type = other RNA; note = The nucleotide modifications are shown in Table 1B
tacaactttcctgaaatgcag

SEQ ID NO: 377 - RNA, 21 nt, synthetic construct
  source 1..21: mol_type = other RNA; note = The nucleotide modifications are shown in Table 1B
tccccatacaactttcctgaa

SEQ ID NO: 378 - RNA, 21 nt, synthetic construct
  source 1..21: mol_type = other RNA; note = The nucleotide modifications are shown in Table 1B
ttccccatacaactttcctga

SEQ ID NO: 379 - RNA, 21 nt, synthetic construct
  source 1..21: mol_type = other RNA; note = The nucleotide modifications are shown in Table 1B
atgatgtcagcagttccccat

SEQ ID NO: 380 - RNA, 21 nt, synthetic construct
  source 1..21: mol_type = other RNA; note = The nucleotide modifications are shown in Table 1B
tcatgatgtcagcagttcccc

SEQ ID NO: 381 - RNA, 21 nt, synthetic construct
  source 1..21: mol_type = other RNA; note = The nucleotide modifications are shown in Table 1B
atcatgatgtcagcagttccc

SEQ ID NO: 382 - RNA, 21 nt, synthetic construct
  source 1..21: mol_type = other RNA; note = The nucleotide modifications are shown in Table 1B
aagccaatcatgatgtcagca

SEQ ID NO: 383 - RNA, 21 nt, synthetic construct
  source 1..21: mol_type = other RNA; note = The nucleotide modifications are shown in Table 1B
tgagccagcgtgtttcctggc

SEQ ID NO: 384 - RNA, 21 nt, synthetic construct
  source 1..21: mol_type = other RNA; note = The nucleotide modifications are shown in Table 1B
aaaggcatgagccagcgtgtt

SEQ ID NO: 385 - RNA, 21 nt, synthetic construct
  source 1..21: mol_type = other RNA; note = The nucleotide modifications are shown in Table 1B
ttcatcctcatcgaagtgagc

SEQ ID NO: 386 - RNA, 21 nt, synthetic construct
  source 1..21: mol_type = other RNA; note = The nucleotide modifications are shown in Table 1B
atccgtccagcgttcatcctc

SEQ ID NO: 387 - RNA, 21 nt, synthetic construct
  source 1..21: mol_type = other RNA; note = The nucleotide modifications are shown in Table 1B
tagactgctaccatccgtcca

SEQ ID NO: 388 - RNA, 21 nt, synthetic construct
  source 1..21: mol_type = other RNA; note = The nucleotide modifications are shown in Table 1B
tttaaaattttggggatctcc

SEQ ID NO: 389 - RNA, 21 nt, synthetic construct
  source 1..21: mol_type = other RNA; note = The nucleotide modifications are shown in Table 1B
aaagtttaaaattttggggat

SEQ ID NO: 390 - RNA, 21 nt, synthetic construct
  source 1..21: mol_type = other RNA; note = The nucleotide modifications are shown in Table 1B
taaagtttaaaattttgggga

SEQ ID NO: 391 - RNA, 21 nt, synthetic construct
  source 1..21: mol_type = other RNA; note = The nucleotide modifications are shown in Table 1B
tatcatcctgggaaagtttaa

SEQ ID NO: 392 - RNA, 21 nt, synthetic construct
  source 1..21: mol_type = other RNA; note = The nucleotide modifications are shown in Table 1B
tctgaatgcctttaatatcat

SEQ ID NO: 393 - RNA, 21 nt, synthetic construct
  source 1..21: mol_type = other RNA; note = The nucleotide modifications are shown in Table 1B
ttctgaatgcctttaatatca

SEQ ID NO: 394 - RNA, 21 nt, synthetic construct
  source 1..21: mol_type = other RNA; note = The nucleotide modifications are shown in Table 1B
tttctgaatgcctttaatatc

SEQ ID NO: 395 - RNA, 21 nt, synthetic construct
  source 1..21: mol_type = other RNA; note = The nucleotide modifications are shown in Table 1B
tttccatatagtttctgaatg

SEQ ID NO: 396 - RNA, 21 nt, synthetic construct
  source 1..21: mol_type = other RNA; note = The nucleotide modifications are shown in Table 1B
tctttccatatagtttctgaa

SEQ ID NO: 397 - RNA, 21 nt, synthetic construct
  source 1..21: mol_type = other RNA; note = The nucleotide modifications are shown in Table 1B
tctctttccatatagtttctg

SEQ ID NO: 398 - RNA, 21 nt, synthetic construct
  source 1..21: mol_type = other RNA; note = The nucleotide modifications are shown in Table 1B
ttctctttccatatagtttct

SEQ ID NO: 399 - RNA, 21 nt, synthetic construct
  source 1..21: mol_type = other RNA; note = The nucleotide modifications are shown in Table 1B
tacttctctttccatatagtt

SEQ ID NO: 400 - RNA, 21 nt, synthetic construct
  source 1..21: mol_type = other RNA; note = The nucleotide modifications are shown in Table 1B
attacttctctttccatatag

SEQ ID NO: 401 - RNA, 21 nt, synthetic construct
  source 1..21: mol_type = other RNA; note = The nucleotide modifications are shown in Table 1B
tgaattacttctctttccata

SEQ ID NO: 402 - RNA, 21 nt, synthetic construct
  source 1..21: mol_type = other RNA; note = The nucleotide modifications are shown in Table 1B
ttgaattacttctctttccat

SEQ ID NO: 403 - RNA, 21 nt, synthetic construct
  source 1..21: mol_type = other RNA; note = The nucleotide modifications are shown in Table 1B
tcttgaattacttctctttcc

SEQ ID NO: 404 - RNA, 21 nt, synthetic construct
  source 1..21: mol_type = other RNA; note = The nucleotide modifications are shown in Table 1B
ttcttgaattacttctctttc

SEQ ID NO: 405 - RNA, 21 nt, synthetic construct
  source 1..21: mol_type = other RNA; note = The nucleotide modifications are shown in Table 1B
tttcttgaattacttctcttt

SEQ ID NO: 406 - RNA, 21 nt, synthetic construct
  source 1..21: mol_type = other RNA; note = The nucleotide modifications are shown in Table 1B
ttttcttgaattacttctctt

SEQ ID NO: 407 - RNA, 21 nt, synthetic construct
  source 1..21: mol_type = other RNA; note = The nucleotide modifications are shown in Table 1B
tctttcttgaattacttctct

SEQ ID NO: 408 - RNA, 21 nt, synthetic construct
  source 1..21: mol_type = other RNA; note = The nucleotide modifications are shown in Table 1B
ttctttcttgaattacttctc

SEQ ID NO: 409 - RNA, 21 nt, synthetic construct
  source 1..21: mol_type = other RNA; note = The nucleotide modifications are shown in Table 1B
tttctttcttgaattacttct

SEQ ID NO: 410 - RNA, 21 nt, synthetic construct
  source 1..21: mol_type = other RNA; note = The nucleotide modifications are shown in Table 1B
tatttctttcttgaattactt

SEQ ID NO: 411 - RNA, 21 nt, synthetic construct
  source 1..21: mol_type = other RNA; note = The nucleotide modifications are shown in Table 1B
tctatttctttcttgaattac

SEQ ID NO: 412 - RNA, 21 nt, synthetic construct
  source 1..21: mol_type = other RNA; note = The nucleotide modifications are shown in Table 1B
agtttctatttctttcttgaa

SEQ ID NO: 413 - RNA, 21 nt, synthetic construct
  source 1..21: mol_type = other RNA; note = The nucleotide modifications are shown in Table 1B
taagtttctatttctttcttg

SEQ ID NO: 414 - RNA, 21 nt, synthetic construct
  source 1..21: mol_type = other RNA; note = The nucleotide modifications are shown in Table 1B
tgaagtttctatttctttctt

SEQ ID NO: 415 - RNA, 21 nt, synthetic construct
  source 1..21: mol_type = other RNA; note = The nucleotide modifications are shown in Table 1B
tgattgtgcaacaatgatata

SEQ ID NO: 416 - RNA, 21 nt, synthetic construct
  source 1..21: mol_type = other RNA; note = The nucleotide modifications are shown in Table 1B
tctgattgtgcaacaatgata

SEQ ID NO: 417 - RNA, 21 nt, synthetic construct
  source 1..21: mol_type = other RNA; note = The nucleotide modifications are shown in Table 1B
aaaagggtgacataattgcta

SEQ ID NO: 418 - RNA, 21 nt, synthetic construct
  source 1..21: mol_type = other RNA; note = The nucleotide modifications are shown in Table 1B
aaaggagtgaaagacattcaa

SEQ ID NO: 419 - RNA, 21 nt, synthetic construct
  source 1..21: mol_type = other RNA; note = The nucleotide modifications are shown in Table 1B
aacatttattgacatctaccc

SEQ ID NO: 420 - RNA, 21 nt, synthetic construct
  source 1..21: mol_type = other RNA; note = The nucleotide modifications are shown in Table 1B
ttaacatttattgacatctac

SEQ ID NO: 421 - RNA, 21 nt, synthetic construct
  source 1..21: mol_type = other RNA; note = The nucleotide modifications are shown in Table 1B
aacattttatttatttgtgta

SEQ ID NO: 422 - RNA, 21 nt, synthetic construct
  source 1..21: mol_type = other RNA; note = The nucleotide modifications are shown in Table 1B
aaacattttatttatttgtgt

SEQ ID NO: 423 - RNA, 21 nt, synthetic construct
  source 1..21: mol_type = other RNA; note = The nucleotide modifications are shown in Table 1B
ataaacattttatttatttgt

SEQ ID NO: 424 - RNA, 21 nt, synthetic construct
  source 1..21: mol_type = other RNA; note = The nucleotide modifications are shown in Table 1B
tggaataaacattttatttat

SEQ ID NO: 425 - RNA, 19 nt, synthetic construct
  source 1..19: mol_type = other RNA; note = The nucleotide modifications are shown in Table 3, with a ligand linked to the 5' end
tgggtagatgtcaataaat

SEQ ID NO: 426 - RNA, 19 nt, synthetic construct
  source 1..19: mol_type = other RNA; note = The nucleotide modifications are shown in Table 3, with a ligand linked to the 5' end
tgactcagaaacaaaaaat

SEQ ID NO: 427 - RNA, 19 nt, synthetic construct
  source 1..19: mol_type = other RNA; note = The nucleotide modifications are shown in Table 3, with a ligand linked to the 5' end
attcaagaaagaaatagaa